European Patent Application EP 4 796 129 A1, published August 26, 2026. Title: Anti-Nectin-4 Antibody-Drug Conjugates Containing Camptothecin Derivatives. Applicant: CELLTRION, INC. The sequence listing filed with the application follows.

SEQUENCE LISTING (14 sequences)

SEQ ID NO: 1 - protein, 5 aa, synthetic construct
SYNMN

SEQ ID NO: 2 - protein, 17 aa, synthetic construct
YISSSSSTIYYADSVKG

SEQ ID NO: 3 - protein, 8 aa, synthetic construct
AYYYGMDV

SEQ ID NO: 4 - protein, 11 aa, synthetic construct
RASQGISGWLA

SEQ ID NO: 5 - protein, 7 aa, synthetic construct
AASTLQS

SEQ ID NO: 6 - protein, 9 aa, synthetic construct
QQANSFPPT

SEQ ID NO: 7 - protein, 117 aa, synthetic construct
EVQLVESGGGLVQPGGSLRLSCAASGFTFSSYNMNWVRQAPGKGLEWVSYISSSSSTIYYADSVKGRFTISRDNAKNSLSLQMNSLRDEDTAVYYCARAYYYGMDVWGQGTTVTVSS

SEQ ID NO: 8 - protein, 107 aa, synthetic construct
DIQMTQSPSSVSASVGDRVTITCRASQGISGWLAWYQQKPGKAPKFLIYAASTLQSGVPSRFSGSGSGTDFTLTISSLQPEDFATYYCQQANSFPPTFGGGTKVEIK

SEQ ID NO: 9 - protein, 447 aa, synthetic construct
EVQLVESGGGLVQPGGSLRLSCAASGFTFSSYNMNWVRQAPGKGLEWVSYISSSSSTIYYADSVKGRFTISRDNAKNSLSLQMNSLRDEDTAVYYCARAYYYGMDVWGQGTTVTVSSASTKGPSVFPLAPSSKSTSGGTAALGCLVKDYFPEPVTVSWNSGALTSGVHTFPAVLQSSGLYSLSSVVTVPSSSLGTQTYICNVNHKPSNTKVDKRVEPKSCDKTHTCPPCPAPELLGGPSVFLFPPKPKDTLMISRTPEVTCVVVDVSHEDPEVKFNWYVDGVEVHNAKTKPREEQYNSTYRVVSVLTVLHQDWLNGKEYKCKVSNKALPAPIEKTISKAKGQPREPQVYTLPPSREEMTKNQVSLTCLVKGFYPSDIAVEWESNGQPENNYKTTPPVLDSDGSFFLYSKLTVDKSRWQQGNVFSCSVMHEALHNHYTQKSLSLSPGK

SEQ ID NO: 10 - protein, 214 aa, synthetic construct
DIQMTQSPSSVSASVGDRVTITCRASQGISGWLAWYQQKPGKAPKFLIYAASTLQSGVPSRFSGSGSGTDFTLTISSLQPEDFATYYCQQANSFPPTFGGGTKVEIKRTVAAPSVFIFPPSDEQLKSGTASVVCLLNNFYPREAKVQWKVDNALQSGNSQESVTEQDSKDSTYSLSSTLTLSKADYEKHKVYACEVTHQGLSSPVTKSFNRGEC

SEQ ID NO: 11 - protein, 449 aa, synthetic construct
EVQLVQSGGGLIQPGGSLRLSCAASEFIVSSNYMTWVRQAPGKGLEWVSIIYPGGSTYYADSVKGRFTISRDNSKNTLYLRMNSLRAEDTAVYYCARDLPLTGTTLDYWGQGTLVTVSSASTKGPSVFPLAPSSKSTSGGTAALGCLVKDYFPEPVTVSWNSGALTSGVHTFPAVLQSSGLYSLSSVVTVPSSSLGTQTYICNVNHKPSNTKVDKRVEPKSCDKTHTCPPCPAPELLGGPSVFLFPPKPKDTLMISRTPEVTCVVVDVSHEDPEVKFNWYVDGVEVHNAKTKPREEQYNSTYRVVSVLTVLHQDWLNGKEYKCKVSNKALPAPIEKTISKAKGQPREPQVYTLPPSRDELTKNQVSLTCLVKGFYPSDIAVEWESNGQPENNYKTTPPVLDSDGSFFLYSKLTVDKSRWQQGNVFSCSVMHEALHNHYTQKSLSLSPGK

SEQ ID NO: 12 - protein, 214 aa, synthetic construct
ELVLTQSPSSLSASVGDRVTITCRASQSISSYLNWYQQKPGKAPKLLIYAASSLQSGVPSRFSGSGSGTDFTLTISSLQPEDFATYYCQQSYSTPLTFGGGTKLEIKRTVAAPSVFIFPPSDEQLKSGTASVVCLLNNFYPREAKVQWKVDNALQSGNSQESVTEQDSKDSTYSLSSTLTLSKADYEKHKVYACEVTHQGLSSPVTKSFNRGEC

SEQ ID NO: 13 - protein, 475 aa, synthetic construct
MDWTWSILFLVAAATGAHSQVQLVQSGAEVKKPGASVKVSCKTSGYSFSTYGVSWVRQAPGQGPEWVGWISAYTGITDYAQKFQGRVTLTTDATTATAFLDLRSLRPDDTATYFCARDKVQGRVEVGSGGRHDYWGQGTLVIVSSASTKGPSVFPLAPSSKSTSGGTAALGCLVKDYFPEPVTVSWNSGALTSGVHTFPAVLQSSGLYSLSSVVTVPSSSLGTQTYICNVNHKPSNTKVDKKVEPKSCDKTHTCPPCPAPELLGGPSVFLFPPKPKDTLMISRTPEVTCVVVDVSHEDPEVKFNWYVDGVEVHNAKTKPREEQYNSTYRVVSVLTVLHQDWLNGKEYKCKVSNKALPAPIEKTISKAKGQPREPQVYTLPPSRDELTKNQVSLTCLVKGFYPSDIAVEWESNGQPENNYKTTPPVLDSDGSFFLYSKLTVDKSRWQQGNVFSCSVMHEGLHNHYTQKSLSLSPGK

SEQ ID NO: 14 - protein, 235 aa, synthetic construct
METPAQLLFLLLLWLPDTTGEVVLTQSPGTLALPPGERATLSCRASHRVGSTYIAWYQQKSGQAPRRLIYGASNRATDIPDRFSGSGSGTDFTLTIRRLEPEDSAVYYCQQFSVSPWTFGQGTRVEIKRTVAAPSVFIFPPSDEQLKSGTASVVCLLNNFYPREAKVQWKVDNALQSGNSQESVTEQDSKDSTYSLSSTLTLSKADYEKHKVYACEVTHQGLSSPVTKSFNRGEC